European Patent Application EP 4 534 553 A1, published April 9, 2025. Title: HUMAN AMYLIN ANALOG, AND DERIVATIVE THEREOF AND USE THEREOF. Applicant: Hang Zhou Sciwind Biosciences Co., Ltd. Application CN PCT/CN2023/096811, filed May 29, 2023. The sequence listing filed with the application follows.

SEQUENCE LISTING (104 sequences)

SEQ ID NO: 1 - protein, 37 aa, synthetic construct
KCNTATCATQRLAEFLRHSSNNFGPILPPTNVGSNTP

SEQ ID NO: 2 - protein, 37 aa, synthetic construct
  MOD_RES 37: note = trans-Hyp-NH2
KCNTATCATQRLADFLRHSSNNLGPILPPTNVGSNTX

SEQ ID NO: 3 - protein, 37 aa, synthetic construct
  MOD_RES 37: note = trans-Hyp-NH2
KCNTATCATQRLADFLRHSSNNLKPILPPTNVGSNTX

SEQ ID NO: 4 - protein, 37 aa, synthetic construct
  MOD_RES 37: note = trans-Hyp-NH2
RCNTATCATQRLADFLRHSKNNLGPILPPTNVGSNTX

SEQ ID NO: 5 - protein, 37 aa, synthetic construct
RCNTATCATQRLAEFLRHSSKNLGPILPPTNVGSNTP

SEQ ID NO: 6 - protein, 37 aa, synthetic construct
RCNTATCATQRLAEFLRHSSNKLGPILPPTNVGSNTP

SEQ ID NO: 7 - protein, 37 aa, synthetic construct
RCNTATCATQRLAEFLRHSSNNKGPILPPTNVGSNTP

SEQ ID NO: 8 - protein, 37 aa, synthetic construct
RCNTATCATQRLAEFLRHSSNNLKPILPPTNVGSNTP

SEQ ID NO: 9 - protein, 37 aa, synthetic construct
RCNTATCATQRLAEFLRHSSNNLGKILPPTNVGSNTP

SEQ ID NO: 10 - protein, 37 aa, synthetic construct
RCNTATCATQRLAEFLRHSSNNLKPILSSTNVGSNTP

SEQ ID NO: 11 - protein, 37 aa, synthetic construct
RCNTATCATQRLAEFLRHSSNNLKAILPSTNVGSNTP

SEQ ID NO: 12 - protein, 37 aa, synthetic construct
RCNTATCATQRLAEFLRHSSNNLKAILSPTNVGSNTP

SEQ ID NO: 13 - protein, 37 aa, synthetic construct
RCNTATCATQRLAEFLRHSSNNLKPILPSTNVGSNTP

SEQ ID NO: 14 - protein, 37 aa, synthetic construct
RCNTATCATQRLAEFLRHSSNNLKPILSPTNVGSNTP

SEQ ID NO: 15 - protein, 37 aa, synthetic construct
RCNTATCATQRLAEFLRHSSNNLKAILPPTNVGSNTP

SEQ ID NO: 16 - protein, 37 aa, synthetic construct
RCNTATCATQRLAEFLRHSSNNLKPILPPTNVGSNTY

SEQ ID NO: 17 - protein, 37 aa, synthetic construct
RCNTATCATQRLAEFLRHSSNNLKAILSSTNVGSNTY

SEQ ID NO: 18 - protein, 37 aa, synthetic construct
RCNTATCATQRLAEFLRHSSNNLKPILSSTNVGSNTY

SEQ ID NO: 19 - protein, 37 aa, synthetic construct
RCNTATCATQRLAEFLRHSSNNLKAILPSTNVGSNTY

SEQ ID NO: 20 - protein, 37 aa, synthetic construct
RCNTATCATQRLAEFLRHSSNNLKAILSPTNVGSNTY

SEQ ID NO: 21 - protein, 37 aa, synthetic construct
RCNTATCATQRLAEFLRHSSNNLKPILPSTNVGSNTY

SEQ ID NO: 22 - protein, 37 aa, synthetic construct
RCNTATCATQRLAEFLRHSSNNLKPILSPTNVGSNTY

SEQ ID NO: 23 - protein, 37 aa, synthetic construct
RCNTATCATQRLAEFLRHSSNNLKAILPPTNVGSNTY

SEQ ID NO: 24 - protein, 37 aa, synthetic construct
RCNTATCATQRLAEFLRHSSNNLKPILPPTNVGSGTP

SEQ ID NO: 25 - protein, 37 aa, synthetic construct
RCNTATCATQRLAEFLRHSSNNLKAILSSTNVGSGTP

SEQ ID NO: 26 - protein, 37 aa, synthetic construct
RCNTATCATQRLAEFLRHSSNNLKPILSSTNVGSGTP

SEQ ID NO: 27 - protein, 37 aa, synthetic construct
RCNTATCATQRLAEFLRHSSNNLKAILPSTNVGSGTP

SEQ ID NO: 28 - protein, 37 aa, synthetic construct
RCNTATCATQRLAEFLRHSSNNLKAILSPTNVGSGTP

SEQ ID NO: 29 - protein, 37 aa, synthetic construct
RCNTATCATQRLAEFLRHSSNNLKPILPSTNVGSGTP

SEQ ID NO: 30 - protein, 37 aa, synthetic construct
RCNTATCATQRLAEFLRHSSNNLKPILSPTNVGSGTP

SEQ ID NO: 31 - protein, 37 aa, synthetic construct
RCNTATCATQRLAEFLRHSSNNLKAILPPTNVGSGTP

SEQ ID NO: 32 - protein, 37 aa, synthetic construct
KCNTATCATQRLAEFLRHSSNNLKPILPPTNVGSNTP

SEQ ID NO: 33 - protein, 37 aa, synthetic construct
KCNTATCATQRLAEFLRHSSNNLKPILSSTNVGSNTP

SEQ ID NO: 34 - protein, 37 aa, synthetic construct
KCNTATCATQRLAEFLRHSSNNLKAILPSTNVGSNTP

SEQ ID NO: 35 - protein, 37 aa, synthetic construct
KCNTATCATQRLAEFLRHSSNNLKAILSPTNVGSNTP

SEQ ID NO: 36 - protein, 37 aa, synthetic construct
KCNTATCATQRLAEFLRHSSNNLKPILPSTNVGSNTP

SEQ ID NO: 37 - protein, 37 aa, synthetic construct
KCNTATCATQRLAEFLRHSSNNLKPILSPTNVGSNTP

SEQ ID NO: 38 - protein, 37 aa, synthetic construct
KCNTATCATQRLAEFLRHSSNNLKAILPPTNVGSNTP

SEQ ID NO: 39 - protein, 37 aa, synthetic construct
  MOD_RES 37: note = trans-Hyp-NH2
RCNTATCATQRLAEFLRHSSNNLKPILPPTNVGSNTX

SEQ ID NO: 40 - protein, 37 aa, synthetic construct
  MOD_RES 37: note = trans-Hyp-NH2
RCNTATCATQRLAEFLRHSSNNLKPILPPTNVGSGTX

SEQ ID NO: 41 - protein, 37 aa, synthetic construct
RCNTATCATQRLADFLRHSSNNLKPILPPTNVGSNTP

SEQ ID NO: 42 - protein, 37 aa, synthetic construct
  MOD_RES 14: note = Aad
RCNTATCATQRLAXFLRHSSNNLKPILPPTNVGSNTP

SEQ ID NO: 43 - protein, 37 aa, synthetic construct; identical to SEQ ID NO: 42
  MOD_RES 14: note = Dab

SEQ ID NO: 44 - protein, 37 aa, synthetic construct; identical to SEQ ID NO: 42
  MOD_RES 14: note = Dap

SEQ ID NO: 45 - protein, 37 aa, synthetic construct
  MOD_RES 17: note = Orn
RCNTATCATQRLAEFLXHSSNNLKPILPPTNVGSNTP

SEQ ID NO: 46 - protein, 37 aa, synthetic construct; identical to SEQ ID NO: 8

SEQ ID NO: 47 - protein, 37 aa, synthetic construct; identical to SEQ ID NO: 41

SEQ ID NO: 48 - protein, 36 aa, synthetic construct
CNTATCATQRLAEFLRHSSNNLKPILPPTNVGSNTP

SEQ ID NO: 49 - protein, 36 aa, synthetic construct
CNTATCATQRLADFLRHSSNNLKPILPPTNVGSNTP

SEQ ID NO: 50 - protein, 37 aa, synthetic construct
  MOD_RES 37: note = trans-Hyp-NH2
RCNTATCATQRLADFLRHSSNNLKPILPPTNVGSNTX

SEQ ID NO: 51 - protein, 36 aa, synthetic construct
  MOD_RES 36: note = trans-Hyp-NH2
CNTATCATQRLAEFLRHSSNNLKPILPPTNVGSNTX

SEQ ID NO: 52 - protein, 36 aa, synthetic construct
  MOD_RES 36: note = trans-Hyp-NH2
CNTATCATQRLADFLRHSSNNLKPILPPTNVGSNTX

SEQ ID NO: 53 - protein, 37 aa, synthetic construct; identical to SEQ ID NO: 39
  MOD_RES 37: note = cis-Hyp-NH2

SEQ ID NO: 54 - protein, 37 aa, synthetic construct; identical to SEQ ID NO: 50
  MOD_RES 37: note = cis-Hyp-NH2

SEQ ID NO: 55 - protein, 37 aa, synthetic construct; identical to SEQ ID NO: 39
  MOD_RES 37: note = Pip-NH2

SEQ ID NO: 56 - protein, 37 aa, synthetic construct; identical to SEQ ID NO: 50
  MOD_RES 37: note = Pip-NH2

SEQ ID NO: 57 - protein, 37 aa, synthetic construct; identical to SEQ ID NO: 39
  MOD_RES 37: note = Aze-NH2

SEQ ID NO: 58 - protein, 37 aa, synthetic construct; identical to SEQ ID NO: 50
  MOD_RES 37: note = Aze-NH2

SEQ ID NO: 59 - protein, 37 aa, synthetic construct; identical to SEQ ID NO: 39
  MOD_RES 37: note = 3-Am-Pro-NH2

SEQ ID NO: 60 - protein, 37 aa, synthetic construct; identical to SEQ ID NO: 50
  MOD_RES 37: note = 3-Am-Pro-NH2

SEQ ID NO: 61 - protein, 37 aa, synthetic construct; identical to SEQ ID NO: 39
  MOD_RES 37: note = alpha MePro-NH2

SEQ ID NO: 62 - protein, 37 aa, synthetic construct; identical to SEQ ID NO: 50
  MOD_RES 37: note = alpha MePro-NH2

SEQ ID NO: 63 - protein, 37 aa, synthetic construct
  MOD_RES 37: note = trans-Hyp-NH2
KCNTATCATQRLADFLRHSSNNFGPILPPTNVGSNTX

SEQ ID NO: 64 - protein, 37 aa, synthetic construct
  MOD_RES 1: note = Dap
  MOD_RES 37: note = trans-Hyp-NH2
XCNTATCATQRLADFLRHSSNNLKPILPPTNVGSNTX

SEQ ID NO: 65 - protein, 37 aa, synthetic construct; identical to SEQ ID NO: 64
  MOD_RES 1: note = Dab
  MOD_RES 37: note = trans-Hyp-NH2

SEQ ID NO: 66 - protein, 37 aa, synthetic construct; identical to SEQ ID NO: 64
  MOD_RES 1: note = Orn
  MOD_RES 37: note = trans-Hyp-NH2

SEQ ID NO: 67 - protein, 37 aa, synthetic construct; identical to SEQ ID NO: 64
  MOD_RES 1: note = Har
  MOD_RES 37: note = trans-Hyp-NH2

SEQ ID NO: 68 - protein, 37 aa, synthetic construct
  MOD_RES 37: note = trans-Hyp-NH2
HCNTATCATQRLADFLRHSSNNLKPILPPTNVGSNTX

SEQ ID NO: 69 - protein, 37 aa, synthetic construct
  MOD_RES 37: note = trans-Hyp-NH2
DCNTATCATQRLADFLRHSSNNLKPILPPTNVGSNTX

SEQ ID NO: 70 - protein, 37 aa, synthetic construct
  METAL 37: note = trans-Hyp-NH2
ECNTATCATQRLADFLRHSSNNLKPILPPTNVGSNTX

SEQ ID NO: 71 - protein, 37 aa, synthetic construct
  MOD_RES 37: note = trans-Hyp-NH2
RCNTATCATQRLADFLRHSSNNKGPILPPTNVGSNTX

SEQ ID NO: 72 - protein, 37 aa, synthetic construct
  MOD_RES 37: note = trans-Hyp-NH2
RCNTATCATQRLADFLRHSSNKLGPILPPTNVGSNTX

SEQ ID NO: 73 - protein, 37 aa, synthetic construct
  MOD_RES 37: note = trans-Hyp-NH2
RCNTATCATQRLADFLRHSSKNLGPILPPTNVGSNTX

SEQ ID NO: 74 - protein, 37 aa, synthetic construct
  MOD_RES 37: note = trans-Hyp-NH2
RCNTATCATQRLADFLRHKSNNLGPILPPTNVGSNTX

SEQ ID NO: 75 - protein, 37 aa, synthetic construct
  MOD_RES 37: note = trans-Hyp-NH2
RCNTATCATQRLADFLRHSSNNLGKILPPTNVGSNTX

SEQ ID NO: 76 - protein, 37 aa, synthetic construct
  MOD_RES 37: note = trans-Hyp-NH2
RCNTATCATQRLADFLRHSSNNLGPILPPTNVGSNTX

SEQ ID NO: 77 - protein, 37 aa, synthetic construct
  MOD_RES 37: note = trans-Hyp-NH2
HCNTATCATQRLADFLRHSSNNLGPILPPTNVGSNTX

SEQ ID NO: 78 - protein, 37 aa, synthetic construct
KCNTATCATQRLANFLVHSSNNFGPILPPTNVGSNTY

SEQ ID NO: 79 - protein, 37 aa, synthetic construct; identical to SEQ ID NO: 3
  MOD_RES 37: note = Aze-NH2

SEQ ID NO: 80 - protein, 37 aa, synthetic construct; identical to SEQ ID NO: 3
  MOD_RES 37: note = Aze-NH2

SEQ ID NO: 81 - protein, 37 aa, synthetic construct; identical to SEQ ID NO: 78

SEQ ID NO: 82 - protein, 37 aa, synthetic construct; identical to SEQ ID NO: 3
  MOD_RES 37: note = Aze-NH2

SEQ ID NO: 83 - protein, 37 aa, synthetic construct
  MOD_RES 37: note = trans-Hyp-NH2
KCNTATCATQRLADFLRHSSNNLRPILPPTNVGSNTX

SEQ ID NO: 84 - protein, 37 aa, synthetic construct
  MOD_RES 37: note = trans-Hyp-NH2
KCNTATCATQRLADFLRHSSNNLHPILPPTNVGSNTX

SEQ ID NO: 85 - protein, 37 aa, synthetic construct
KCNTATCATQRLADFLRHSSNNLKPILPPTNVGSNTP

SEQ ID NO: 86 - protein, 37 aa, synthetic construct
KCNTATCATQRLADFLRHSSNNLRPILPPTNVGSNTP

SEQ ID NO: 87 - protein, 37 aa, synthetic construct
KCNTATCATQRLADFLRHSSNNLHPILPPTNVGSNTP

SEQ ID NO: 88 - protein, 37 aa, synthetic construct
KCNTATCATQRLADFLRHSSNNLPPILPPTNVGSNTP

SEQ ID NO: 89 - protein, 37 aa, synthetic construct
KCNTATCATQRLADFLRHSSNNLDPILPPTNVGSNTP

SEQ ID NO: 90 - protein, 37 aa, synthetic construct
KCNTATCATQRLADFLRHSSNNLNPILPPTNVGSNTP

SEQ ID NO: 91 - protein, 37 aa, synthetic construct
KCNTATCATQRLADFLRHSSNNLSPILPPTNVGSNTP

SEQ ID NO: 92 - protein, 37 aa, synthetic construct
  MOD_RES 24: note = alpha K
KCNTATCATQRLADFLRHSSNNLXPILPPTNVGSNTP

SEQ ID NO: 93 - protein, 37 aa, synthetic construct; identical to SEQ ID NO: 92
  MOD_RES 24: note = Dap

SEQ ID NO: 94 - protein, 37 aa, synthetic construct; identical to SEQ ID NO: 92
  MOD_RES 24: note = Dab

SEQ ID NO: 95 - protein, 37 aa, synthetic construct; identical to SEQ ID NO: 92
  MOD_RES 24: note = Orn

SEQ ID NO: 96 - protein, 37 aa, synthetic construct; identical to SEQ ID NO: 92
  MOD_RES 24: note = Cit

SEQ ID NO: 97 - protein, 37 aa, synthetic construct; identical to SEQ ID NO: 92
  MOD_RES 24: note = Sar

SEQ ID NO: 98 - protein, 37 aa, synthetic construct; identical to SEQ ID NO: 92
  MOD_RES 24: note = Trx

SEQ ID NO: 99 - protein, 37 aa, synthetic construct; identical to SEQ ID NO: 92
  MOD_RES 24: note = AOC

SEQ ID NO: 100 - protein, 37 aa, synthetic construct; identical to SEQ ID NO: 2
  MOD_RES 37: note = Aze-NH2

SEQ ID NO: 101 - protein, 37 aa, synthetic construct; identical to SEQ ID NO: 3
  MOD_RES 37: note = trans-Hyp-NH2

SEQ ID NO: 102 - protein, 37 aa, synthetic construct; identical to SEQ ID NO: 85

SEQ ID NO: 103 - protein, 37 aa, synthetic construct
RCNTATCATQRLADFLRHSSNNLRPILPPTNVGSNTP

SEQ ID NO: 104 - protein, 42 aa, synthetic construct
KGGGGRCNTATCATQRLADFLRHSSNNLRPILPPTNVGSNTP